European Patent Application EP 4 659 807 A2, published December 10, 2025. Title: ANTIBODIES BINDING TO CITRULLINATED HISTONE 2A AND/OR 4. Applicant: Citryll B.V. Application EP, filed August 20, 2019. The sequence listing filed with the application follows.

SEQUENCE LISTING (56 sequences)

SEQ ID NO: 1 - protein, 8 aa, synthetic construct
  REGION 1..8: note = CDR1 of msVH22.101 and hVH22.101(HC)x
GYTFTNYG

SEQ ID NO: 2 - protein, 8 aa, synthetic construct
  REGION 1..8: note = CDR2 of msVH22.101 and hVH22.101(HC)x
INTYSGEA

SEQ ID NO: 3 - protein, 15 aa, synthetic construct
  REGION 1..15: note = CDR3 of msVH22.101 and hVH22.101(HC)x
LRGYTYQSFDEGGDY

SEQ ID NO: 4 - skipped

SEQ ID NO: 5 - protein, 9 aa, synthetic construct
  REGION 1..9: note = CDR3 of msVL22.101 and hVL22.101(LC)y
WQGTHFPYT

SEQ ID NO: 6 - protein, 11 aa, Homo sapiens
QSLLDTDGKTY

SEQ ID NO: 7 - protein, 11 aa, Homo sapiens
QSLLDSDAKTY

SEQ ID NO: 8 - protein, 11 aa, Homo sapiens
QSLLDTDAKTY

SEQ ID NO: 9 - protein, 11 aa, Homo sapiens
QSLLDADGKTY

SEQ ID NO: 10 - protein, 11 aa, Homo sapiens
QSLLDNDGKTY

SEQ ID NO: 11 - protein, 122 aa, synthetic construct
  REGION 1..122: note = hVH22.101f
RIQLVQSGAEVKKPGASVKVSCKASGYTFTNYGMHWVRQAPGQGLEWMGWINTYSGEATYAQKFQGRVTMTRDTSISTAYMELSRLRSDDTAVYYCLRGYTYQSFDEGGDYWGQGTLVTVSS

SEQ ID NO: 12 - protein, 122 aa, Homo sapiens
RIQLVQSGAEVKKPGASVKVSCKASGYTFTNYGMHWVRQAPGQGLEWMGWINTYSGEATYVDDFQGRVTMTRDTSISTAYMELSRLRSDDTAVYYCLRGYTYQSFDEGGDYWGQGTLVTVSS

SEQ ID NO: 13 - protein, 112 aa, Homo sapiens
DVVMTQSPLSLPVTLGQPASISCRSSQSLLDTDGKTYLNWFQQRPGQSPRRLIYLVSKLDSGVPDRFSGSGSGTDFTLKISRVEAEDVGVYYCWQGTHFPYTFGQGTKLEIK

SEQ ID NO: 14 - protein, 112 aa, Homo sapiens
DVVMTQSPLSLPVTLGQPASISCRSSQSLLDSDAKTYLNWFQQRPGQSPRRLIYLVSKLDSGVPDRFSGSGSGTDFTLKISRVEAEDVGVYYCWQGTHFPYTFGQGTKLEIK

SEQ ID NO: 15 - protein, 112 aa, Homo sapiens
DVVMTQSPLSLPVTLGQPASISCRSSQSLLDTDAKTYLNWFQQRPGQSPRRLIYLVSKLDSGVPDRFSGSGSGTDFTLKISRVEAEDVGVYYCWQGTHFPYTFGQGTKLEIK

SEQ ID NO: 16 - protein, 112 aa, Homo sapiens
DVVMTQSPLSLPVTLGQPASISCRSSQSLLDADGKTYLNWFQQRPGQSPRRLIYLVSKLDSGVPDRFSGSGSGTDFTLKISRVEAEDVGVYYCWQGTHFPYTFGQGTKLEIK

SEQ ID NO: 17 - protein, 112 aa, Homo sapiens
DVVMTQSPLSLPVTLGQPASISCRSSQSLLDNDGKTYLNWFQQRPGQSPRRLIYLVSKLDSGVPDRFSGSGSGTDFTLKISRVEAEDVGVYYCWQGTHFPYTFGQGTKLEIK

SEQ ID NO: 18 - protein, 12 aa, Homo sapiens
  MOD_RES 3: note = citrulline
SGRGKQGGKARA

SEQ ID NO: 19 - protein, 23 aa, Homo sapiens
  MOD_RES 3: note = citrulline
SGRGKGGKGLGKGGAKRHRKVLR

SEQ ID NO: 20 - protein, 12 aa, Homo sapiens
  MOD_RES 3: note = citrulline
SGRGKGGKGLGK

SEQ ID NO: 21 - protein, 12 aa, Homo sapiens
  MOD_RES 6: note = citrulline
QFPVGRVHRLLR

SEQ ID NO: 22 - protein, 12 aa, Homo sapiens
  MOD_RES 6: note = citrulline
VHRLLRKGNYSE

SEQ ID NO: 23 - protein, 329 aa, Homo sapiens
ASTKGPSVFPLAPSSKSTSGGTAALGCLVKDYFPEPVTVSWNSGALTSGVHTFPAVLQSSGLYSLSSVVTVPSSSLGTQTYICNVNHKPSNTKVDKKVEPKSCDKTHTCPPCPAPELLGGPSVFLFPPKPKDTLMISRTPEVTCVVVDVSHEDPEVKFNWYVDGVEVHNAKTKPREEQYNSTYRVVSVLTVLHQDWLNGKEYKCKVSNKALPAPIEKTISKAKGQPREPQVYTLPPSRDELTKNQVSLTCLVKGFYPSDIAVEWESNGQPENNYKTTPPVLDSDGSFFLYSKLTVDKSRWQQGNVFSCSVMHEALHNHYTQKSLSLSPG

SEQ ID NO: 24 - protein, 107 aa, Homo sapiens [sequence omitted]

SEQ ID NO: 25 - protein, 122 aa, Mus musculus
RIQLVQSGPELKKPGEAVKISCKASGYTFTNYGMHWMKQTPGKDFRWMGWINTYSGEATYVDDFKGRFAFSLGTSASTAYLQINNLKNDDTATYFCLRGYTYQSFDEGGDYWGQGTALTVSS

SEQ ID NO: 26 - protein, 122 aa, Homo sapiens
QVQLVQSGAEVKKPGASVKVSCKASGYTFTNYGMHWVRQAPGQGLEWMGWINTYSGEATYAQKFQGRVTMTRDTSISTAYMELSRLRSDDTAVYYCLRGYTYQSFDEGGDYWGQGTLVTVSS

SEQ ID NO: 27 - protein, 122 aa, Homo sapiens
QVQLVQSGAEVKKPGSSVKVSCKASGYTFTNYGMHWVRQAPGQGLEWMGWINTYSGEATYAQKFQGRVTITADESTSTAYMELSSLRSEDTAVYYCLRGYTYQSFDEGGDYWGQGTLVTVSS

SEQ ID NO: 28 - protein, 122 aa, Homo sapiens
QVQLVQSGAEVKKPGSSVKVSCKASGYTFTNYGMHWVRQAPGQGLEWMGWINTYSGEATYVDDFQGRVTITADESTSTAYMELSSLRSEDTAVYYCLRGYTYQSFDEGGDYWGQGTLVTVSS

SEQ ID NO: 29 - protein, 122 aa, Homo sapiens
QVQLVQSGAEVKKPGASVKVSCKASGYTFTNYGMHWVRQAPGQGLEWMGWINTYSGEATYVDDFQGRVTMTRDTSISTAYMELSRLRSDDTAVYYCLRGYTYQSFDEGGDYWGQGTLVTVSS

SEQ ID NO: 30 - protein, 112 aa, Mus musculus
DVVMTQTPLTLSVTTGQPASISCKSSQSLLDSDGKTYLNWLFQRPGQSPKRLIYLVSKLDSGVPDRFTGSGSGTDFTLKISRVEAEDLGIYYCWQGTHFPYTFGGGTNLEIK

SEQ ID NO: 31 - protein, 112 aa, Homo sapiens
DVVMTQSPLSLPVTLGQPASISCRSSQSLVDSDGKTYLNWFQQRPGQSPRRLIYLVSKLDSGVPDRFSGSGSGTDFTLKISRVEAEDVGVYYCWQGTHFPYTFGQGTKLEIK

SEQ ID NO: 32 - protein, 112 aa, Homo sapiens
DVVMTQSPLSLPVTLGQPASISCRSSQSLLDSDGKTYLNWFQQRPGQSPRRLIYLVSKLDSGVPDRFSGSGSGTDFTLKISRVEAEDVGVYYCWQGTHFPYTFGQGTKLEIK

SEQ ID NO: 33 - protein, 112 aa, Homo sapiens
DVVMTQSPLSLPVTLGQPASISCRSSQSLVASDGKTYLNWFQQRPGQSPRRLIYLVSKLDSGVPDRFSGSGSGTDFTLKISRVEAEDVGVYYCWQGTHFPYTFGQGTKLEIK

SEQ ID NO: 34 - protein, 112 aa, Homo sapiens
DVVMTQSPLSLPVTLGQPASISCRSSQSLVESDGKTYLNWFQQRPGQSPRRLIYLVSKLDSGVPDRFSGSGSGTDFTLKISRVEAEDVGVYYCWQGTHFPYTFGQGTKLEIK

SEQ ID NO: 35 - protein, 112 aa, Homo sapiens
DVVMTQSPLSLPVTLGQPASISCRSSQSLVSSDGKTYLNWFQQRPGQSPRRLIYLVSKLDSGVPDRFSGSGSGTDFTLKISRVEAEDVGVYYCWQGTHFPYTFGQGTKLEIK

SEQ ID NO: 36 - protein, 11 aa, synthetic construct
  REGION 1..11: note = CDR1 of msVL22.101 and hVL22.101g
QSLLDSDGKTY

SEQ ID NO: 37 - protein, 11 aa, Homo sapiens
QSLVDSDGKTY

SEQ ID NO: 38 - protein, 11 aa, Homo sapiens
QSLVASDGKTY

SEQ ID NO: 39 - protein, 11 aa, Homo sapiens
QSLVESDGKTY

SEQ ID NO: 40 - protein, 11 aa, Homo sapiens
QSLVSSDGKTY

SEQ ID NO: 41 - protein, 11 aa, Homo sapiens
QSLLESDGKTY

SEQ ID NO: 42 - protein, 11 aa, Homo sapiens
QSLLDSEGKTY

SEQ ID NO: 43 - protein, 11 aa, Homo sapiens
QSLLDSSGKTY

SEQ ID NO: 44 - protein, 11 aa, Homo sapiens
QSLLESEGKTY

SEQ ID NO: 45 - protein, 11 aa, Homo sapiens
QSLLESSGKTY

SEQ ID NO: 46 - protein, 11 aa, Homo sapiens
QSLLESDAKTY

SEQ ID NO: 47 - protein, 11 aa, Homo sapiens
QSLLDTEGKTY

SEQ ID NO: 48 - protein, 11 aa, Homo sapiens
QSLLDTSGKTY

SEQ ID NO: 49 - protein, 11 aa, Homo sapiens
QSLLDSAGKTY

SEQ ID NO: 50 - protein, 11 aa, Homo sapiens
QSLLESAGKTY

SEQ ID NO: 51 - protein, 11 aa, Homo sapiens
QSLLDAEGKTY

SEQ ID NO: 52 - protein, 11 aa, Homo sapiens
QSLLDNEGKTY

SEQ ID NO: 53 - protein, 17 aa, Homo sapiens
  MOD_RES 9: note = citrulline
EPTDSLDARGHRPVDRR

SEQ ID NO: 54 - protein, 15 aa, Homo sapiens
  MOD_RES 4: note = citrulline
  MOD_RES 9: note = citrulline
  MOD_RES 11: note = citrulline
YVTRSSAVRLRSSVP

SEQ ID NO: 55 - protein, 7 aa, synthetic construct
  REGION 1..7: note = Region around CDR2 of msVL22.101 and hVL22.101(LC)y
LVSKLDS

SEQ ID NO: 56 - protein, 330 aa, Homo sapiens [sequence omitted]